European Patent Application EP 4 502 164 A1, published February 5, 2025. Title: Glucose-Regulated Gene Expression Loop Control System and Use Thereof in Regulating and Controlling Blood Glucose. Applicant: East China Normal University. The sequence listing filed with the application follows.

SEQUENCE LISTING (80 sequences)

SEQ ID NO: 1 - DNA, 64 bp, synthetic construct
  source 1..64: mol_type = other DNA
ttgacatcccacctcacgtatgctataatgtgtgcagtctgacgcggcgttgttggaattacaa

SEQ ID NO: 2 - DNA, 79 bp, synthetic construct
  source 1..79: mol_type = other DNA
ttgacatcccacctcacgtatgctataatgtgtgcagtctgacgcggcgttgttggaattacaattgttggaattacaa

SEQ ID NO: 3 - DNA, 94 bp, synthetic construct
  source 1..94: mol_type = other DNA
ttgacatcccacctcacgtatgctataatgtgtgcagtctgacgcggcgttgttggaattacaattgttggaattacaattgttggaattacaa

SEQ ID NO: 4 - DNA, 109 bp, synthetic construct
  source 1..109: mol_type = other DNA
ttgacatcccacctcacgtatgctataatgtgtgcagtctgacgcggcgttgttggaattacaattgttggaattacaattgttggaattacaattgttggaattacaa

SEQ ID NO: 5 - DNA, 124 bp, synthetic construct
  source 1..124: mol_type = other DNA
ttgacatcccacctcacgtatgctataatgtgtgcagtctgacgcggcgttgttggaattacaattgttggaattacaattgttggaattacaattgttggaattacaattgttggaattacaa

SEQ ID NO: 6 - DNA, 91 bp, synthetic construct
  source 1..91: mol_type = other DNA
tttacactttatgcttccggctcgtatgttgttgttggaattacaattgttggaattacaattgttggaattacaattgttggaattacaa

SEQ ID NO: 7 - DNA, 81 bp, synthetic construct
  source 1..81: mol_type = other DNA
tttacactttatgcttccggctcgtatgttggtgtgcagtctgacgcggcgttgttggaattacaattgttggaattacaa

SEQ ID NO: 8 - DNA, 96 bp, synthetic construct
  source 1..96: mol_type = other DNA
tttacactttatgcttccggctcgtatgttggtgtgcagtctgacgcggcgttgttggaattacaattgttggaattacaattgttggaattacaa

SEQ ID NO: 9 - DNA, 111 bp, synthetic construct
  source 1..111: mol_type = other DNA
tttacactttatgcttccggctcgtatgttggtgtgcagtctgacgcggcgttgttggaattacaattgttggaattacaattgttggaattacaattgttggaattacaa

SEQ ID NO: 10 - DNA, 126 bp, synthetic construct
  source 1..126: mol_type = other DNA
tttacactttatgcttccggctcgtatgttggtgtgcagtctgacgcggcgttgttggaattacaattgttggaattacaattgttggaattacaattgttggaattacaattgttggaattacaa

SEQ ID NO: 11 - protein, 31 aa, synthetic construct
HSEGTFTSDVSSYLEGQAAQEFIAWLVNGRG

SEQ ID NO: 12 - protein, 36 aa, synthetic construct
DDDDKHSEGTFTSDVSSYLEGQAAQEFIAWLVNGRG

SEQ ID NO: 13 - protein, 270 aa, synthetic construct
HSEGTFTSDVSSYLEGQAAQEFIAWLVNGRGGGGGSISAMVRSDKTHTCPPCPAPELLGGPSVFLFPPKPKDTLMISRTPEVTCVVVDVSHEDPEVKFNWYVDGVEVHNAKTKPREEQYNSTYRVVSVLTVLHQDWLNGKEYKCKVSNKALPAPIEKTISKAKGQPREPQVYTLPPSREEMTKNQVSLTCLVKGFYPSDIAVEWESNGQPENNYKTTPPVLDSDGSFFLYSKLTVDKSRWQQGNVFSCSVMHEALHNHYTQKSLSLSPGK

SEQ ID NO: 14 - protein, 136 aa, synthetic construct
MANYKKPKLLYCSNGGHFLRILPDGTVDGTRDRSDQHIQLQLSAESVGEVYIKSTETGQYLAMDTDGLLYGSQTPNEECLFLERLEENHYNTYISKKHAEKNWFVGLKKNGSCKRGPRTHYGQKAILFLPLPVSSD

SEQ ID NO: 15 - protein, 69 aa, synthetic construct
MKPVSLSYRCPCRFFESHVARANVKHLKILNTPNCALQIVARLKNNNRQVCIDPKLKWIQEYLEKALNK

SEQ ID NO: 16 - DNA, 35 bp, synthetic construct
  source 1..35: mol_type = other DNA
ttgttggaattacaacccctctagaaataattttg

SEQ ID NO: 17 - DNA, 35 bp, synthetic construct
  source 1..35: mol_type = other DNA
ttgtaattccaacaacgccgcgtcagactgcacac

SEQ ID NO: 18 - DNA, 48 bp, synthetic construct
  source 1..48: mol_type = other DNA
ggagaaatactagatggcagatcttgtgcgaaacctcctggaacagat

SEQ ID NO: 19 - DNA, 46 bp, synthetic construct
  source 1..46: mol_type = other DNA
tttctttaccagactcgagggtacctcagttgaggtcgtcgtcctc

SEQ ID NO: 20 - DNA, 50 bp, synthetic construct
  source 1..50: mol_type = other DNA
ttgtaattccaacaattgtaattccaacaacgccgcgtcagactgcacac

SEQ ID NO: 21 - DNA, 50 bp, synthetic construct
  source 1..50: mol_type = other DNA
ttgttggaattacaattgttggaattacaacccctctagaaataattttg

SEQ ID NO: 22 - DNA, 80 bp, synthetic construct
  source 1..80: mol_type = other DNA
ttgtaattccaacaattgtaattccaacaattgtaattccaacaattgtaattccaacaacgccgcgtcagactgcacac

SEQ ID NO: 23 - DNA, 65 bp, synthetic construct
  source 1..65: mol_type = other DNA
ttgtaattccaacaattgtaattccaacaattgttggaattacaacccctctagaaataattttg

SEQ ID NO: 24 - DNA, 54 bp, synthetic construct
  source 1..54: mol_type = other DNA
tttacactttatgcttccggctcgtatgttggtgtgcagtctgacgcggcgttg

SEQ ID NO: 25 - DNA, 50 bp, synthetic construct
  source 1..50: mol_type = other DNA
cggaagcataaagtgtaaacttaagcatatggtgcactctcagtacaatc

SEQ ID NO: 26 - DNA, 48 bp, synthetic construct
  source 1..48: mol_type = other DNA
tttgtttaactttaagaaggagatataccgtgcgaaacctcctggaac

SEQ ID NO: 27 - DNA, 57 bp, synthetic construct
  source 1..57: mol_type = other DNA
tctccttcttaaagttaaacaaaattatttctagacattatacgagccgatgattaa

SEQ ID NO: 28 - DNA, 45 bp, synthetic construct
  source 1..45: mol_type = other DNA
gactcgtcttataaggaaagttaacggtgcgaaacctcctggaac

SEQ ID NO: 29 - DNA, 53 bp, synthetic construct
  source 1..53: mol_type = other DNA
gttaactttccttataagacgagtctattcattatacgagccgatgattaatt

SEQ ID NO: 30 - DNA, 45 bp, synthetic construct
  source 1..45: mol_type = other DNA
acaacaaagcaaaaatagggggttcggtgcgaaacctcctggaac

SEQ ID NO: 31 - DNA, 51 bp, synthetic construct
  source 1..51: mol_type = other DNA
aaccccctatttttgctttgttgtgctcattatacgagccgatgattaatt

SEQ ID NO: 32 - DNA, 60 bp, synthetic construct
  source 1..60: mol_type = other DNA
ttaagaaggagatataccatgggcagcagcatgactaaaaaaatttcattcattattaac

SEQ ID NO: 33 - DNA, 50 bp, synthetic construct
  source 1..50: mol_type = other DNA
agcttgtcgacggagctcgaattctcaactattaaatgcttggtttaagc

SEQ ID NO: 34 - DNA, 68 bp, synthetic construct
  source 1..68: mol_type = other DNA
tgctctggctctgctgccgctgctgtttaccccggtaaccaaggcacattccgaaggcacctttacct

SEQ ID NO: 35 - DNA, 52 bp, synthetic construct
  source 1..52: mol_type = other DNA
agaaggagatataccatgatgaaacagtccaccattgctctggctctgctgc

SEQ ID NO: 36 - DNA, 40 bp, synthetic construct
  source 1..40: mol_type = other DNA
tgctcgagtgcggccgctcacttgtcatcgtcatccttgt

SEQ ID NO: 37 - DNA, 56 bp, synthetic construct
  source 1..56: mol_type = other DNA
tgcactggctggtttcgcgaccgtggcacaggctcattccgaaggcacctttacct

SEQ ID NO: 38 - DNA, 65 bp, synthetic construct
  source 1..65: mol_type = other DNA
agaaggagatataccatgatgaaaaaaaccgctatcgcaatcgccgttgcactggctggtttcgc

SEQ ID NO: 39 - DNA, 61 bp, synthetic construct
  source 1..61: mol_type = other DNA
atagtactaacgaccccgattgcgattagctcttttgcgcatagcgaaggcaccttcacct

SEQ ID NO: 40 - DNA, 59 bp, synthetic construct
  source 1..59: mol_type = other DNA
agaaggagatataccatgagggctaaattattgggaatagtactaacgaccccgattgc

SEQ ID NO: 41 - DNA, 57 bp, synthetic construct
  source 1..57: mol_type = other DNA
tagcggtggctgtggcggcgggtgttatgagcgcacaggcacatagcgagggcacct

SEQ ID NO: 42 - DNA, 60 bp, synthetic construct
  source 1..60: mol_type = other DNA
agaaggagatataccatgatgataacattgaggaaattacccctagcggtggctgtggcg

SEQ ID NO: 43 - DNA, 56 bp, synthetic construct
  source 1..56: mol_type = other DNA
tgcgggcctgttgttgctggctgcgcagccggcaatggcgcatagcgagggcacct

SEQ ID NO: 44 - DNA, 58 bp, synthetic construct
  source 1..58: mol_type = other DNA
agaaggagatataccatgaaatatttactacccacagcagctgcgggcctgttgttgc

SEQ ID NO: 45 - DNA, 56 bp, synthetic construct
  source 1..56: mol_type = other DNA
aagctttatatctacaagtttgccgctgccgacccatagcgaaggtacgtttacct

SEQ ID NO: 46 - DNA, 51 bp, synthetic construct
  source 1..51: mol_type = other DNA
agaaggagatataccatgaaaatttcaagctttatatctacaagtttgccg

SEQ ID NO: 47 - DNA, 42 bp, synthetic construct
  source 1..42: mol_type = other DNA
ccgaccgacgacgacgacaagcatagcgaaggtacgtttacc

SEQ ID NO: 48 - DNA, 39 bp, synthetic construct
  source 1..39: mol_type = other DNA
cgctatgcttgtcgtcgtcgtcggtcggcagcggcaaac

SEQ ID NO: 49 - DNA, 42 bp, synthetic construct; identical to SEQ ID NO: 47
  source 1..42: mol_type = other DNA

SEQ ID NO: 50 - DNA, 36 bp, synthetic construct
  source 1..36: mol_type = other DNA
tggtggtgctcgagtttacccggagacagggagagg

SEQ ID NO: 51 - DNA, 25 bp, synthetic construct
  source 1..25: mol_type = other DNA
taaactcgagcaccaccaccaccac

SEQ ID NO: 52 - DNA, 39 bp, synthetic construct; identical to SEQ ID NO: 48
  source 1..39: mol_type = other DNA

SEQ ID NO: 53 - DNA, 64 bp, synthetic construct
  source 1..64: mol_type = other DNA
agcagctttattagtaccagtctgccgctgccgaccgctaactataaaaaaccgaaactgctgt

SEQ ID NO: 54 - DNA, 52 bp, synthetic construct
  source 1..52: mol_type = other DNA
ttaagaaggagatataccatgaagatcagcagctttattagtaccagtctgc

SEQ ID NO: 55 - DNA, 65 bp, synthetic construct
  source 1..65: mol_type = other DNA
gtcgacggagctcgaattcttaagcgtaatctggaacatcgtatgggtagtccgacgacaccggc

SEQ ID NO: 56 - DNA, 76 bp, synthetic construct
  source 1..76: mol_type = other DNA
atagcgattgctgtagcgctggcgggttttgctaccgttgctcaggcgaaaccggtgagtctgagttatcgttgcc

SEQ ID NO: 57 - DNA, 58 bp, synthetic construct
  source 1..58: mol_type = other DNA
taactttaagaaggagatataccatgaaaaagacagcaatagcgattgctgtagcgct

SEQ ID NO: 58 - DNA, 79 bp, synthetic construct
  source 1..79: mol_type = other DNA
gtcgacggagctcgaattcttaagcgtaatctggaacatcgtatgggtatttattcagtgctttttccagatattcctg

SEQ ID NO: 59 - DNA, 74 bp, synthetic construct
  source 1..74: mol_type = other DNA
attacgcttaagaattcaatagactcgtcttataaggaaagttaacgatgaaaaagacagcaatagcgattgct

SEQ ID NO: 60 - DNA, 47 bp, synthetic construct
  source 1..47: mol_type = other DNA
tggtggtggtggtgctcgagtttattcagtgctttttccagatattc

SEQ ID NO: 61 - protein, 284 aa, synthetic construct
MNSEEQYYAATQLYKDPCAFQRGPVPEFSANPPACLYMGRQPPPPPPPQFTSSLGSLEQGSPPDISPYEVPPLASDDPAGAHLHHHLPAQLGLAHPPPGPFPNGTEPGGLEEPNRVQLPFPWMKSTKAHAWKGQWAGGAYTAEPEENKRTRTAYTRAQLLELEKEFLFNKYISRPRRVELAVMLNLTERHIKIWFQNRRMKWKKEEDKKRSSGTPSGGGGGEEPEQDCAVTSGEELLAVPPLPPPGGAVPPGVPAAVREGLLPSGLSVSPQPSSIAPLRPQEPR

SEQ ID NO: 62 - DNA, 39 bp, synthetic construct
  source 1..39: mol_type = other DNA
caccaccaccaccaccacatgaacagtgaggagcagtac

SEQ ID NO: 63 - DNA, 61 bp, synthetic construct
  source 1..61: mol_type = other DNA
ttaacgacgacgctggcggcgttttttacggccgtaaccgccaccccggggttcctgcggt

SEQ ID NO: 64 - DNA, 38 bp, synthetic construct
  source 1..38: mol_type = other DNA
gccagcgtcgtcgttaatgagatccggctgctaacaaa

SEQ ID NO: 65 - DNA, 34 bp, synthetic construct
  source 1..34: mol_type = other DNA
tggtggtggtggtggtgggtcggcagcggcaaac

SEQ ID NO: 66 - protein, 283 aa, synthetic construct
MNGEEQYYAATQLYKDPCAFQRGPAPEFSASPPACLYMGRQPPPPPPHPFPGALGALEQGSPPDISPYEVPPLADDPAVAHLHHHLPAQLALPHPPAGPFPEGAEPGVLEEPNRVQLPFPWMKSTKAHAWKGQWAGGAYAAEPEENKRTRTAYTRAQLLELEKEFLFNKYISRPRRVELAVMLNLTERHIKIWFQNRRMKWKKEEDKKRGGGTAVGGGGVAEPEQDCAVTSGEELLALPPPPPPGGAVPPAAPVAAREGRLPPGLSASPQPSSVAPRRPQEPR

SEQ ID NO: 67 - DNA, 37 bp, synthetic construct
  source 1..37: mol_type = other DNA
caccaccaccaccaccacatgaacggcgaggagcagt

SEQ ID NO: 68 - DNA, 62 bp, synthetic construct
  source 1..62: mol_type = other DNA
ttaacgacgacgctggcggcgttttttacggccgtaaccgccacctcgtggttcctgcggcc

SEQ ID NO: 69 - DNA, 38 bp, synthetic construct; identical to SEQ ID NO: 64
  source 1..38: mol_type = other DNA

SEQ ID NO: 70 - DNA, 34 bp, synthetic construct; identical to SEQ ID NO: 65
  source 1..34: mol_type = other DNA

SEQ ID NO: 71 - DNA, 70 bp, synthetic construct
  source 1..70: mol_type = other DNA
atccggctgctaacaaaggaaataattttgtttaactttaagaaggagatataccatgaaaatttcaagc

SEQ ID NO: 72 - DNA, 39 bp, synthetic construct
  source 1..39: mol_type = other DNA
caactcagcttcctttcgggttaacgacgacgctggcgg

SEQ ID NO: 73 - DNA, 22 bp, synthetic construct
  source 1..22: mol_type = other DNA
aaggaagctgagttggctgctg

SEQ ID NO: 74 - DNA, 24 bp, synthetic construct
  source 1..24: mol_type = other DNA
tcctttgttagcagccggatctca

SEQ ID NO: 75 - protein, 129 aa, synthetic construct [sequence omitted]

SEQ ID NO: 76 - DNA, 49 bp, synthetic construct
  source 1..49: mol_type = other DNA
ggaagatcttccaaagaggagaaatactagatgaaaatctcctctttca

SEQ ID NO: 77 - DNA, 33 bp, synthetic construct
  source 1..33: mol_type = other DNA
cggggtaccccgccggatctcagtggtggtggt

SEQ ID NO: 78 - DNA, 15 bp, synthetic construct
  source 1..15: mol_type = other DNA
ttgtggtttttacta

SEQ ID NO: 79 - DNA, 15 bp, synthetic construct
  source 1..15: mol_type = other DNA
ttgtaattccaacaa

SEQ ID NO: 80 - DNA, 16 bp, synthetic construct
  source 1..16: mol_type = other DNA
ttgtttaaatatacaa